European Patent Application EP 4 389 215 A1, published June 26, 2024. Title: Chemically modified TDP-43 derived polypeptides and uses thereof. Applicant: CONSEJO SUPERIOR DE INVESTIGACIONES CIENTIFICAS (CSIC). The sequence listing filed with the application follows.

SEQUENCE LISTING (15 sequences)

SEQ ID NO: 1 - protein, 42 aa, Homo sapiens
GGMNFGAFSINPAMMAAAQAALQSSWGMMGMLASQQNQSGPS

SEQ ID NO: 2 - protein, 141 aa, Homo sapiens
GRFGGNPGGFGNQGGFGNSRGGGAGLGNNQGSNMGGGMNFGAFSINPAMMAAAQAALQSSWGMMGMLASQQNQSGPSGNNQNQGNMQREPNQAFGSGNNSYSGSNSGAAIGWGSASNAGSGSGFNGGFGSSMDSKSSGWGM

SEQ ID NO: 3 - protein, 414 aa, Homo sapiens
MSEYIRVTEDENDEPIEIPSEDDGTVLLSTVTAQFPGACGLRYRNPVSQCMRGVRLVEGILHAPDAGWGNLVYVVNYPKDNKRKMDETDASSAVKVKRAVQKTSDLIVLGLPWKTTEQDLKEYFSTFGEVLMVQVKKDLKTGHSKGFGFVRFTEYETQVKVMSQRHMIDGRWCDCKLPNSKQSQDEPLRSRKVFVGRCTEDMTEDELREFFSQYGDVMDVFIPKPFRAFAFVTFADDQIAQSLCGEDLIIKGISVHISNAEPKHNSNRQLERSGRFGGNPGGFGNQGGFGNSRGGGAGLGNNQGSNMGGGMNFGAFSINPAMMAAAQAALQSSWGMMGMLASQQNQSGPSGNNQNQGNMQREPNQAFGSGNNSYSGSNSGAAIGWGSASNAGSGSGFNGGFGSSMDSKSSGWGM

SEQ ID NO: 4 - DNA, 31 bp, synthetic construct
  source 1..31: mol_type = other DNA
atttccagggatccatgtctgaatatattcg

SEQ ID NO: 5 - DNA, 32 bp, synthetic construct
  source 1..32: mol_type = other DNA
gtggtgctcgagttacattccccagccagaag

SEQ ID NO: 6 - DNA, 21 bp, synthetic construct
  source 1..21: mol_type = other DNA
ctcgagcaccaccaccaccac

SEQ ID NO: 7 - DNA, 29 bp, synthetic construct
  source 1..29: mol_type = other DNA
gacatggatccctggaaatacaggttttc

SEQ ID NO: 8 - DNA, 33 bp, synthetic construct
  source 1..33: mol_type = other DNA
atttccagggatccggaagatttggtggtaatc

SEQ ID NO: 9 - DNA, 32 bp, synthetic construct; identical to SEQ ID NO: 5
  source 1..32: mol_type = other DNA

SEQ ID NO: 10 - DNA, 21 bp, synthetic construct
  source 1..21: mol_type = other DNA
ctcgagcaccaccaccaccac

SEQ ID NO: 11 - DNA, 29 bp, synthetic construct
  source 1..29: mol_type = other DNA
cttccggatccctggaaatacaggttttc

SEQ ID NO: 12 - DNA, 21 bp, synthetic construct
  source 1..21: mol_type = other DNA
ctcgagcaccaccaccaccac

SEQ ID NO: 13 - DNA, 29 bp, synthetic construct
  source 1..29: mol_type = other DNA
gaaaacctgtatttccagggatccggtgg

SEQ ID NO: 14 - DNA, 30 bp, synthetic construct
  source 1..30: mol_type = other DNA
atttccagggatccggtgggatgaactttg

SEQ ID NO: 15 - DNA, 28 bp, synthetic construct
  source 1..28: mol_type = other DNA
cagtcaggcccatcgtaactcgagcacc